European Patent Application EP 4 257 686 A1, published October 11, 2023. Title: Asymmetric nucleic acid molecules inducing RNA interference that Inhibits Expression of ROR-beta. Applicant: OliX Pharmaceuticals, Inc. Konkuk University Glocal Industry-Academic Collaboration Foundation. The sequence listing filed with the application follows.

SEQUENCE LISTING (128 sequences)

SEQ ID NO: 1 - RNA, 16 nt, Artificial Sequence
  asiRORB-001 sense
aaauuuguggcgauaa

SEQ ID NO: 2 - RNA, 19 nt, Artificial Sequence
  asiRORB-001 antisense
uuaucgccacaaauuuugc

SEQ ID NO: 3 - RNA, 16 nt, Artificial Sequence
  asiRORB-002 sense
aaaauuuguggcgaua

SEQ ID NO: 4 - RNA, 19 nt, Artificial Sequence
  asiRORB-002 antisense
uaucgccacaaauuuugca

SEQ ID NO: 5 - RNA, 16 nt, Artificial Sequence
  asiRORB-003 sense
accaugcaaaauuugu

SEQ ID NO: 6 - RNA, 19 nt, Artificial Sequence
  asiRORB-003 antisense
acaaauuuugcaugguauc

SEQ ID NO: 7 - RNA, 16 nt, Artificial Sequence
  asiRORB-004 sense
gauaccaugcaaaauu

SEQ ID NO: 8 - RNA, 19 nt, Artificial Sequence
  asiRORB-004 antisense
aauuuugcaugguaucacu

SEQ ID NO: 9 - RNA, 16 nt, Artificial Sequence
  asiRORB-005 sense
ugauaccaugcaaaau

SEQ ID NO: 10 - RNA, 19 nt, Artificial Sequence
  asiRORB-005 antisense
auuuugcaugguaucacuu

SEQ ID NO: 11 - RNA, 16 nt, Artificial Sequence
  asiRORB-006 sense
gugauaccaugcaaaa

SEQ ID NO: 12 - RNA, 19 nt, Artificial Sequence
  asiRORB-006 antisense
uuuugcaugguaucacuuc

SEQ ID NO: 13 - RNA, 16 nt, Artificial Sequence
  asiRORB-007 sense
agugauaccaugcaaa

SEQ ID NO: 14 - RNA, 19 nt, Artificial Sequence
  asiRORB-007 antisense
uuugcaugguaucacuuca

SEQ ID NO: 15 - RNA, 16 nt, Artificial Sequence
  asiRORB-008 sense
aagugauaccaugcaa

SEQ ID NO: 16 - RNA, 19 nt, Artificial Sequence
  asiRORB-008 antisense
uugcaugguaucacuucaa

SEQ ID NO: 17 - RNA, 16 nt, Artificial Sequence
  asiRORB-009 sense
auugaagugauaccau

SEQ ID NO: 18 - RNA, 19 nt, Artificial Sequence
  asiRORB-009 antisense
augguaucacuucaauuug

SEQ ID NO: 19 - RNA, 16 nt, Artificial Sequence
  asiRORB-010 sense
cacuacggagucauca

SEQ ID NO: 20 - RNA, 19 nt, Artificial Sequence
  asiRORB-010 antisense
ugaugacuccguaguggau

SEQ ID NO: 21 - RNA, 16 nt, Artificial Sequence
  asiRORB-011 sense
uccacuacggagucau

SEQ ID NO: 22 - RNA, 19 nt, Artificial Sequence
  asiRORB-011 antisense
augacuccguaguggaucc

SEQ ID NO: 23 - RNA, 16 nt, Artificial Sequence
  asiRORB-012 sense
auccacuacggaguca

SEQ ID NO: 24 - RNA, 19 nt, Artificial Sequence
  asiRORB-012 antisense
ugacuccguaguggauccc

SEQ ID NO: 25 - RNA, 16 nt, Artificial Sequence
  asiRORB-013 sense
gagccagcagaacaau

SEQ ID NO: 26 - RNA, 19 nt, Artificial Sequence
  asiRORB-013 antisense
auuguucugcuggcuccuc

SEQ ID NO: 27 - RNA, 16 nt, Artificial Sequence
  asiRORB-014 sense
ggagccagcagaacaa

SEQ ID NO: 28 - RNA, 19 nt, Artificial Sequence
  asiRORB-014 antisense
uuguucugcuggcuccucc

SEQ ID NO: 29 - RNA, 16 nt, Artificial Sequence
  asiRORB-015 sense
aggagccagcagaaca

SEQ ID NO: 30 - RNA, 19 nt, Artificial Sequence
  asiRORB-015 antisense
uguucugcuggcuccuccu

SEQ ID NO: 31 - RNA, 16 nt, Artificial Sequence
  asiRORB-016 sense
uguuuaauugacagaa

SEQ ID NO: 32 - RNA, 19 nt, Artificial Sequence
  asiRORB-016 antisense
uucugucaauuaaacaguu

SEQ ID NO: 33 - RNA, 16 nt, Artificial Sequence
  asiRORB-017 sense
cuguuuaauugacaga

SEQ ID NO: 34 - RNA, 19 nt, Artificial Sequence
  asiRORB-017 antisense
ucugucaauuaaacaguuu

SEQ ID NO: 35 - RNA, 16 nt, Artificial Sequence
  asiRORB-018 sense
cugaggugcagaagca

SEQ ID NO: 36 - RNA, 19 nt, Artificial Sequence
  asiRORB-018 antisense
ugcuucugcaccucagcau

SEQ ID NO: 37 - RNA, 16 nt, Artificial Sequence
  asiRORB-019 sense
augcugaggugcagaa

SEQ ID NO: 38 - RNA, 19 nt, Artificial Sequence
  asiRORB-019 antisense
uucugcaccucagcauaca

SEQ ID NO: 39 - RNA, 16 nt, Artificial Sequence
  asiRORB-020 sense
agcagcagagugggga

SEQ ID NO: 40 - RNA, 19 nt, Artificial Sequence
  asiRORB-020 antisense
uccccacucugcugcugcc

SEQ ID NO: 41 - RNA, 16 nt, Artificial Sequence
  asiRORB-021 sense
uguacagcagcagcau

SEQ ID NO: 42 - RNA, 19 nt, Artificial Sequence
  asiRORB-021 antisense
augcugcugcuguacaccc

SEQ ID NO: 43 - RNA, 16 nt, Artificial Sequence
  asiRORB-022 sense
auugaccugcccaagu

SEQ ID NO: 44 - RNA, 19 nt, Artificial Sequence
  asiRORB-022 antisense
acuugggcaggucaaugac

SEQ ID NO: 45 - RNA, 16 nt, Artificial Sequence
  asiRORB-023 sense
acgggcacgucauuga

SEQ ID NO: 46 - RNA, 19 nt, Artificial Sequence
  asiRORB-023 antisense
ucaaugacgugcccguugg

SEQ ID NO: 47 - RNA, 16 nt, Artificial Sequence
  asiRORB-024 sense
uuguuuaccuauagcu

SEQ ID NO: 48 - RNA, 19 nt, Artificial Sequence
  asiRORB-024 antisense
agcuauagguaaacaaguu

SEQ ID NO: 49 - RNA, 16 nt, Artificial Sequence
  asiRORB-025 sense
caacuuguuuaccuau

SEQ ID NO: 50 - RNA, 19 nt, Artificial Sequence
  asiRORB-025 antisense
auagguaaacaaguugggu

SEQ ID NO: 51 - RNA, 16 nt, Artificial Sequence
  asiRORB-026 sense
ccaacuuguuuaccua

SEQ ID NO: 52 - RNA, 19 nt, Artificial Sequence
  asiRORB-026 antisense
uagguaaacaaguugggua

SEQ ID NO: 53 - RNA, 16 nt, Artificial Sequence
  asiRORB-027 sense
uugcacagaacaucau

SEQ ID NO: 54 - RNA, 19 nt, Artificial Sequence
  asiRORB-027 antisense
augauguucugugcaauuc

SEQ ID NO: 55 - RNA, 16 nt, Artificial Sequence
  asiRORB-028 sense
auugcacagaacauca

SEQ ID NO: 56 - RNA, 19 nt, Artificial Sequence
  asiRORB-028 antisense
ugauguucugugcaauucg

SEQ ID NO: 57 - RNA, 16 nt, Artificial Sequence
  asiRORB-029 sense
aaagcaaguccaggga

SEQ ID NO: 58 - RNA, 19 nt, Artificial Sequence
  asiRORB-029 antisense
ucccuggacuugcuuugau

SEQ ID NO: 59 - RNA, 16 nt, Artificial Sequence
  asiRORB-030 sense
uaacaggcuucaugga

SEQ ID NO: 60 - RNA, 19 nt, Artificial Sequence
  asiRORB-030 antisense
uccaugaagccuguuaucc

SEQ ID NO: 61 - RNA, 16 nt, Artificial Sequence
  asiRORB-031 sense
ggauaacaggcuucau

SEQ ID NO: 62 - RNA, 19 nt, Artificial Sequence
  asiRORB-031 antisense
augaagccuguuauccgcu

SEQ ID NO: 63 - RNA, 16 nt, Artificial Sequence
  asiRORB-032 sense
cggauaacaggcuuca

SEQ ID NO: 64 - RNA, 19 nt, Artificial Sequence
  asiRORB-032 antisense
ugaagccuguuauccgcuu

SEQ ID NO: 65 - RNA, 16 nt, Artificial Sequence
  asiRORB-033 sense
gaaaauauggaggaau

SEQ ID NO: 66 - RNA, 19 nt, Artificial Sequence
  asiRORB-033 antisense
auuccuccauauuuuccuu

SEQ ID NO: 67 - RNA, 16 nt, Artificial Sequence
  asiRORB-034 sense
ggaaaauauggaggaa

SEQ ID NO: 68 - RNA, 19 nt, Artificial Sequence
  asiRORB-034 antisense
uuccuccauauuuuccuuc

SEQ ID NO: 69 - RNA, 16 nt, Artificial Sequence
  asiRORB-035 sense
ugaaggaaaauaugga

SEQ ID NO: 70 - RNA, 19 nt, Artificial Sequence
  asiRORB-035 antisense
uccauauuuuccuucaaac

SEQ ID NO: 71 - RNA, 16 nt, Artificial Sequence
  asiRORB-036 sense
cuguuugaaggaaaau

SEQ ID NO: 72 - RNA, 19 nt, Artificial Sequence
  asiRORB-036 antisense
auuuuccuucaaacagaac

SEQ ID NO: 73 - RNA, 16 nt, Artificial Sequence
  asiRORB-037 sense
ucuguuugaaggaaaa

SEQ ID NO: 74 - RNA, 19 nt, Artificial Sequence
  asiRORB-037 antisense
uuuuccuucaaacagaaca

SEQ ID NO: 75 - RNA, 16 nt, Artificial Sequence
  asiRORB-038 sense
uucuguuugaaggaaa

SEQ ID NO: 76 - RNA, 19 nt, Artificial Sequence
  asiRORB-038 antisense
uuuccuucaaacagaacag

SEQ ID NO: 77 - RNA, 16 nt, Artificial Sequence
  asiRORB-039 sense
guucuguuugaaggaa

SEQ ID NO: 78 - RNA, 19 nt, Artificial Sequence
  asiRORB-039 antisense
uuccuucaaacagaacagu

SEQ ID NO: 79 - RNA, 16 nt, Artificial Sequence
  asiRORB-040 sense
cacuguucuguuugaa

SEQ ID NO: 80 - RNA, 19 nt, Artificial Sequence
  asiRORB-040 antisense
uucaaacagaacaguguug

SEQ ID NO: 81 - RNA, 16 nt, Artificial Sequence
  asiRORB-041 sense
acacuguucuguuuga

SEQ ID NO: 82 - RNA, 19 nt, Artificial Sequence
  asiRORB-041 antisense
ucaaacagaacaguguugu

SEQ ID NO: 83 - RNA, 16 nt, Artificial Sequence
  asiRORB-042 sense
caacacuguucuguuu

SEQ ID NO: 84 - RNA, 19 nt, Artificial Sequence
  asiRORB-042 antisense
aaacagaacaguguuguuu

SEQ ID NO: 85 - RNA, 16 nt, Artificial Sequence
  asiRORB-043 sense
acaacacuguucuguu

SEQ ID NO: 86 - RNA, 19 nt, Artificial Sequence
  asiRORB-043 antisense
aacagaacaguguuguuua

SEQ ID NO: 87 - RNA, 16 nt, Artificial Sequence
  asiRORB-044 sense
uaaacaacacuguucu

SEQ ID NO: 88 - RNA, 19 nt, Artificial Sequence
  asiRORB-044 antisense
agaacaguguuguuuaaug

SEQ ID NO: 89 - RNA, 16 nt, Artificial Sequence
  asiRORB-045 sense
uucaaagccuuagguu

SEQ ID NO: 90 - RNA, 19 nt, Artificial Sequence
  asiRORB-045 antisense
aaccuaaggcuuugaacau

SEQ ID NO: 91 - RNA, 16 nt, Artificial Sequence
  asiRORB-046 sense
ugaagcauuugacuuu

SEQ ID NO: 92 - RNA, 19 nt, Artificial Sequence
  asiRORB-046 antisense
aaagucaaaugcuucauuc

SEQ ID NO: 93 - RNA, 16 nt, Artificial Sequence
  asiRORB-047 sense
augaagcauuugacuu

SEQ ID NO: 94 - RNA, 19 nt, Artificial Sequence
  asiRORB-047 antisense
aagucaaaugcuucauuca

SEQ ID NO: 95 - RNA, 16 nt, Artificial Sequence
  asiRORB-048 sense
aaugaagcauuugacu

SEQ ID NO: 96 - RNA, 19 nt, Artificial Sequence
  asiRORB-048 antisense
agucaaaugcuucauucac

SEQ ID NO: 97 - RNA, 16 nt, Artificial Sequence
  asiRORB-049 sense
ugaaugaagcauuuga

SEQ ID NO: 98 - RNA, 19 nt, Artificial Sequence
  asiRORB-049 antisense
ucaaaugcuucauucacua

SEQ ID NO: 99 - RNA, 16 nt, Artificial Sequence
  asiRORB-050 sense
agugaaugaagcauuu

SEQ ID NO: 100 - RNA, 19 nt, Artificial Sequence
  asiRORB-050 antisense
aaaugcuucauucacuagg

SEQ ID NO: 101 - RNA, 16 nt, Artificial Sequence
  asiRORB-051 sense
uagugaaugaagcauu

SEQ ID NO: 102 - RNA, 19 nt, Artificial Sequence
  asiRORB-051 antisense
aaugcuucauucacuaggu

SEQ ID NO: 103 - RNA, 16 nt, Artificial Sequence
  asiRORB-052 sense
cuagugaaugaagcau

SEQ ID NO: 104 - RNA, 19 nt, Artificial Sequence
  asiRORB-052 antisense
augcuucauucacuagguc

SEQ ID NO: 105 - RNA, 16 nt, Artificial Sequence
  asiRORB-053 sense
guuccuugcagcugac

SEQ ID NO: 106 - RNA, 19 nt, Artificial Sequence
  asiRORB-053 antisense
gucagcugcaaggaacaca

SEQ ID NO: 107 - RNA, 16 nt, Artificial Sequence
  asiRORB-054 sense
agaagcuucaggaaaa

SEQ ID NO: 108 - RNA, 19 nt, Artificial Sequence
  asiRORB-054 antisense
uuuuccugaagcuucugga

SEQ ID NO: 109 - RNA, 16 nt, Artificial Sequence
  asiRORB-055 sense
cagaagcuucaggaaa

SEQ ID NO: 110 - RNA, 19 nt, Artificial Sequence
  asiRORB-055 antisense
uuuccugaagcuucuggac

SEQ ID NO: 111 - RNA, 16 nt, Artificial Sequence
  asiRORB-056 sense
augugauucagaagaa

SEQ ID NO: 112 - RNA, 19 nt, Artificial Sequence
  asiRORB-056 antisense
uucuucugaaucacauguu

SEQ ID NO: 113 - RNA, 16 nt, Artificial Sequence
  asiRORB-057 sense
caugugauucagaaga

SEQ ID NO: 114 - RNA, 19 nt, Artificial Sequence
  asiRORB-057 antisense
ucuucugaaucacauguug

SEQ ID NO: 115 - RNA, 16 nt, Artificial Sequence
  asiRORB-058 sense
auagccaagauaccaa

SEQ ID NO: 116 - RNA, 19 nt, Artificial Sequence
  asiRORB-058 antisense
uugguaucuuggcuauuaa

SEQ ID NO: 117 - RNA, 16 nt, Artificial Sequence
  asiRORB-059 sense
guuaauagccaagaua

SEQ ID NO: 118 - RNA, 19 nt, Artificial Sequence
  asiRORB-059 antisense
uaucuuggcuauuaacuuu

SEQ ID NO: 119 - RNA, 16 nt, Artificial Sequence
  asiRORB-060 sense
aguuaauagccaagau

SEQ ID NO: 120 - RNA, 19 nt, Artificial Sequence
  asiRORB-060 antisense
aucuuggcuauuaacuuug

SEQ ID NO: 121 - RNA, 16 nt, Artificial Sequence
  asiRORB-061 sense
aaguuaauagccaaga

SEQ ID NO: 122 - RNA, 19 nt, Artificial Sequence
  asiRORB-061 antisense
ucuuggcuauuaacuuugc

SEQ ID NO: 123 - RNA, 16 nt, Artificial Sequence
  asiRORB-062 sense
gaauacacuguuuccu

SEQ ID NO: 124 - RNA, 19 nt, Artificial Sequence
  asiRORB-062 antisense
aggaaacaguguauucacu

SEQ ID NO: 125 - DNA, 21 bp, Artificial Sequence
  ROR-beta Forward primer
tgcccaagtccgaaggttatt

SEQ ID NO: 126 - DNA, 20 bp, Artificial Sequence
  ROR-beta Reverse primer
ccatgccagctgatggagtt

SEQ ID NO: 127 - DNA, 20 bp, Artificial Sequence
  GAPDH Forward primer
gggtgtgaaccacgagaaat

SEQ ID NO: 128 - DNA, 20 bp, Artificial Sequence
  GAPDH Reverse primer
gtcatgagcccttccacaat